European Patent Specification EP 3 508 212 B1, published October 22, 2025. Title: An Agent for Regeneration of Visual Function or Prevention of Decrease of Visual Function. Applicant: Keio University Nagoya Institute of Technology. The sequence listing filed with the application follows.

SEQUENCE LISTING (9 sequences)

SEQ ID NO: 1 - protein, 317 aa, Artificial Sequence
  Artificial Peptide
MLMTVFSSAPELALLGSTFAQVDPSNLSVSDSLTYGQFNLVYNAFSFAIAAMFASALFFFSAQALVGQRYRLALLVSAIVVSIAGYHYFRIFNSWDAAYVLENGVYSLTSEKFNDAYRYVDWLLTVPLLLVQTVAVIERYVVVCKPMSNFRFGENHPLLIKLTVASVLMIATGYPGEISDDITTRIIWGTVSTIPFAYILYVLWVELSFTVKEAAAQQQESATTQVQTLVRNMRWLLLLSWGVYPIAYLLPMLGVSGTSAAVGVQVGYTIADVLAKPVFGLLVFAIALVKTKADQESSEPHAAIGAAANKSGGSLIS

SEQ ID NO: 2 - protein, 344 aa, Artificial Sequence
  Artificial Peptide
MLMTVFSSAPELALLGSTFAQVDPSNLSVSDSLTYGQFNLVYNAFSFAIAAMFASALFFFSAQALVGQRYRLALLVSAIVVSIAGYHYFRIFNSWDAAYVLENGVYSLTSEKFNDAYRYVDWLLTVPLLLVQTVAVIERYVVVCKPMSNFRFGENHPLLIKLTVASVLMIATGYPGEISDDITTRIIWGTVSTIPFAYILYVLWVELSFTVKEAAAQQQESATTQVQTLVRNMRWLLLLSWGVYPIAYLLPMLGVSGTSAAVGVQVGYTIADVLAKPVFGLLVFAIALVKTKADQESSEPHAAIGAAANKSGGSLISGSASASNGASDYKDDDDKEFFCYENEV

SEQ ID NO: 3 - protein, 344 aa, Artificial Sequence
  Artificial Peptide
MLMTVFSSAPELALLGSTFAQVDPSNLSVSDSLTYGQFNLVYNAFSFAIAAMFASALFFFSAQALVGQRYRLALLVSAIVVSIAGYHYFRIFNSWDAAYVLENGVYSLTSEKFNDAYRYVDWLLTVPLLLVETVAVIERYVVVCKPMSNFRFGENHPLLIKLTVASVLMIATGYPGEISDDITTRIIWGTVSTIPFAYILYVLWVELSFTVKEAAAQQQESATTQVQTLVRNMRWLLLLSWGVYPIAYLLPMLGVSGTSAAVGVQVGYTIADVLAKPVFGLLVFAIALVKTKADQESSEPHAAIGAAANKSGGSLISGSASASNGASDYKDDDDKEFFCYENEV

SEQ ID NO: 4 - protein, 311 aa, Artificial Sequence
  Artificial Peptide
MASQVVYGEWASTHTECYNMSRIDSTFVSLLQLVWAVVSGCQTIFMISRAPKVPWESVYLPFVESITYALASTGNGTLQMRDGRFFPWSRMASWLCTCPIMLGQISNMIERYVVVCKPMSNFRFGENHIPLNPIAQAASIIRVVMGITATISPAEYMKWLFFFFGATCLVFEYSVVFTIFQVGLFTVKEAAAQQQESATTQAQKVVVRIKMLRLIFFIAWTMFPIVWLISPTGVCVIHENVSAILYLLADGLCKNTYGVILWSTAWGVLEGKWDPACLPGQEKPEADDPFGLNHEKNAPPNDEVNIRMFGR

SEQ ID NO: 5 - protein, 11 aa, Artificial Sequence
  Artificial Peptide
IERYVVVCKPM

SEQ ID NO: 6 - protein, 20 aa, Artificial Sequence
  Artificial Peptide
IERYVVVCKPMSNFRFGENH

SEQ ID NO: 7 - protein, 17 aa, Artificial Sequence
  Artificial Peptide
FTVKEAAAQQQESATTQ

SEQ ID NO: 8 - protein, 298 aa, Gloeobacter violaceus
MLMTVFSSAPELALLGSTFAQVDPSNLSVSDSLTYGQFNLVYNAFSFAIAAMFASALFFFSAQALVGQRYRLALLVSAIVVSIAGYHYFRIFNSWDAAYVLENGVYSLTSEKFNDAYRYVDWLLTVPLLLVETVAVLTLPAKEARPLLIKLTVASVLMIATGYPGEISDDITTRIIWGTVSTIPFAYILYVLWVELSRSLVRQPAAVQTLVRNMRWLLLLSWGVYPIAYLLPMLGVSGTSAAVGVQVGYTIADVLAKPVFGLLVFAIALVKTKADQESSEPHAAIGAAANKSGGSLIS

SEQ ID NO: 9 - protein, 348 aa, Bos taurus
MNGTEGPNFYVPFSNKTGVVRSPFEAPQYYLAEPWQFSMLAAYMFLLIMLGFPINFLTLYVTVQHKKLRTPLNYILLNLAVADLFMVFGGFTTTLYTSLHGYFVFGPTGCNLEGFFATLGGEIALWSLVVLAIERYVVVCKPMSNFRFGENHAIMGVAFTWVMALACAAPPLVGWSRYIPEGMQCSCGIDYYTPHEETNNESFVIYMFVVHFIIPLIVIFFCYGQLVFTVKEAAAQQQESATTQKAEKEVTRMVIIMVIAFLICWLPYAGVAFYIFTHQGSDFGPIFMTIPAFFAKTSAVYNPVIYIMMNKQFRNCMVTTLCCGKNPLGDDEASTTVSKTETSQVAPA